European Patent Application EP 4 389 763 A1, published June 26, 2024. Title: FGF21 MUTANT PROTEIN AND USE THEREOF. Applicant: LETO LABORATORIES CO., LTD. The sequence listing filed with the application follows.

SEQUENCE LISTING (27 sequences)

SEQ ID NO: 1 - protein, 181 aa, Homo sapiens
HPIPDSSPLLQFGGQVRQRYLYTDDAQQTEAHLEIREDGTVGGAADQSPESLLQLKALKPGVIQILGVKTSRFLCQRPDGALYGSLHFDPEACSFRELLLEDGYNVYQSEAHGLPLHLPGNKSPHRDPAPRGPARFLPLPGLPPALPEPPGILAPQPPDVGSSDPLSMVGPSQGRSPSYAS

SEQ ID NO: 2 - protein, 182 aa, synthetic construct
  REGION 1..182: note = FGF21 mutant protein 1414
AHPIPDSSPLLQFGGQVRQRYLYTDDAQQTEAHLEIREDGTVGGAADQSPESLLQLKALKPGVIQILGVKTSRFLCQRPDGALYGSLHFDPEACSFRELLLEDGYNVYQSEAHGLPLHLPGQKSPHRDPAPRGPARFLPLPGLPPALPEPPGILAPQPPDVGSSDPLSLVGPSQGRSPSYAS

SEQ ID NO: 3 - protein, 182 aa, synthetic construct
  REGION 1..182: note = FGF21 mutant protein 1407
AHPIPDSSPLLQFGGQVRQRYLYTDDAQQTEAHLEIREDGTVGGAADQSPESLLQLKALKPGVIQILGVKTSRFLCQRPDGALYGSLHFDPEACSFRELLLEDGYNVYQSEAHGLPLHLPGQKSPHRDPAPRGPARFLPLPGLPPALPEPPGILAPQPPDVGSSDPLSLVGGSQGRSPSYAS

SEQ ID NO: 4 - protein, 181 aa, synthetic construct
  REGION 1..181: note = FGF21 mutant protein 1408
AHPIPDSSPLLQFGGQVRQRYLYTDDAQQTEAHLEIREDGTVGGAADQSPESLLQLKALKPGVIQILGVKTSRFLCQRPDGALYGSLHFDPEACSFRELLLEDGYNVYQSEAHGLPLHLPGQKSPHRDPAPRGPARFLPLPGLPPALPEPPGILAPQPPDVGSSDPLSLVGSQGRSPSYAS

SEQ ID NO: 5 - protein, 183 aa, synthetic construct
  REGION 1..183: note = FGF21 mutant protein 1409
AHPIPDSSPLLQFGGQVRQRYLYTDDAQQTEAHLEIREDGTVGGAADQSPESLLQLKALKPGVIQILGVKTSRFLCQRPDGALYGSLHFDPEACSFRELLLEDGYNVYQSEAHGLPLHLPGQKSPHRDPAPRGPARFLPLPGLPPALPEPPGILAPQPPDVGSSDPLSLVCPGCQGRSPSYAS

SEQ ID NO: 6 - protein, 182 aa, synthetic construct
  REGION 1..182: note = FGF21 mutant protein 1410
AHPIPDSSPLLQFGGQVRQRYLYTDDAQQTEAHLEIREDGTVGGAADQSPESLLQLKALKPGVIQILGVKTSRFLCQRPDGALYGSLHFDPEACSFRELLLEDGYNVYQSEAHGLPLHLPGQKSPHRDPAPRGPARFLPLPGLPPALPEPPGILAPQPPDVGSSDPLSLVCPCQGRSPSYAS

SEQ ID NO: 7 - protein, 182 aa, synthetic construct
  REGION 1..182: note = FGF21 mutant protein 1411
AHPIPDSSPLLQFGGQVRQRYLYTDDAQQTEAHLEIREDGTVGGAADQSPESLLQLKALKPGVIQILGVKTSRFLCQRPDGALYGSLHFDPEACSFRELLLEDGYNVYQSEAHGLPLHLPGQKSPHRDPAPRGPARFLPLPGLPPALPEPPGILAPQPPDVGSSDPLSLVCPSCGRSPSYAS

SEQ ID NO: 8 - protein, 183 aa, synthetic construct
  REGION 1..183: note = FGF21 mutant protein 1412
AHPIPDSSPLLQFGGQVRQRYLYTDDAQQTEAHLEIREDGTVGGAADQSPESLLQLKALKPGVIQILGVKTSRFLCQRPDGALYGSLHFDPEACSFRELLLEDGYNVYQSEAHGLPLHLPGQKSPHRDPAPRGPARFLPLPGLPPALPEPPGILAPQPPDVGSSDPLSLVCPACQGRSPSYAS

SEQ ID NO: 9 - protein, 183 aa, synthetic construct
  REGION 1..183: note = FGF21 mutant protein 1413
AHPIPDSSPLLQFGGQVRQRYLYTDDAQQTEAHLEIREDGTVGGAADQSPESLLQLKALKPGVIQILGVKTSRFLCQRPDGALYGSLHFDPEACSFRELLLEDGYNVYQSEAHGLPLHLPGQKSPHRDPAPRGPARFLPLPGLPPALPEPPGILAPQPPDVGSSDPLSLVCPSCQGRSPSYAS

SEQ ID NO: 10 - protein, 180 aa, synthetic construct
  REGION 1..180: note = FGF21 mutant protein
HPIPDSSPLLQFGGQVRQRYLYTDDAQQTEAHLEIREDGTVGGAADQSPESLLQLKALKPGVIQILGVKTSRFLCQRPDGALYGSLHFDPEACSFRELLLEDGYNVYQSEAHGLPLHLPGQKSPHRDPAPRGPARFLPLPGLPPALPEPPGILAPQPPDVGSSDPLSLVGSQGRSPSYAS

SEQ ID NO: 11 - protein, 182 aa, synthetic construct
  REGION 1..182: note = FGF21 mutant protein
HPIPDSSPLLQFGGQVRQRYLYTDDAQQTEAHLEIREDGTVGGAADQSPESLLQLKALKPGVIQILGVKTSRFLCQRPDGALYGSLHFDPEACSFRELLLEDGYNVYQSEAHGLPLHLPGQKSPHRDPAPRGPARFLPLPGLPPALPEPPGILAPQPPDVGSSDPLSLVCPGCQGRSPSYAS

SEQ ID NO: 12 - protein, 181 aa, synthetic construct
  REGION 1..181: note = FGF21 mutant protein
HPIPDSSPLLQFGGQVRQRYLYTDDAQQTEAHLEIREDGTVGGAADQSPESLLQLKALKPGVIQILGVKTSRFLCQRPDGALYGSLHFDPEACSFRELLLEDGYNVYQSEAHGLPLHLPGQKSPHRDPAPRGPARFLPLPGLPPALPEPPGILAPQPPDVGSSDPLSLVCPCQGRSPSYAS

SEQ ID NO: 13 - protein, 181 aa, synthetic construct
  REGION 1..181: note = FGF21 mutant protein
HPIPDSSPLLQFGGQVRQRYLYTDDAQQTEAHLEIREDGTVGGAADQSPESLLQLKALKPGVIQILGVKTSRFLCQRPDGALYGSLHFDPEACSFRELLLEDGYNVYQSEAHGLPLHLPGQKSPHRDPAPRGPARFLPLPGLPPALPEPPGILAPQPPDVGSSDPLSLVCPSCGRSPSYAS

SEQ ID NO: 14 - protein, 182 aa, synthetic construct
  REGION 1..182: note = FGF21 mutant protein
HPIPDSSPLLQFGGQVRQRYLYTDDAQQTEAHLEIREDGTVGGAADQSPESLLQLKALKPGVIQILGVKTSRFLCQRPDGALYGSLHFDPEACSFRELLLEDGYNVYQSEAHGLPLHLPGQKSPHRDPAPRGPARFLPLPGLPPALPEPPGILAPQPPDVGSSDPLSLVCPACQGRSPSYAS

SEQ ID NO: 15 - protein, 182 aa, synthetic construct
  REGION 1..182: note = FGF21 mutant protein
HPIPDSSPLLQFGGQVRQRYLYTDDAQQTEAHLEIREDGTVGGAADQSPESLLQLKALKPGVIQILGVKTSRFLCQRPDGALYGSLHFDPEACSFRELLLEDGYNVYQSEAHGLPLHLPGQKSPHRDPAPRGPARFLPLPGLPPALPEPPGILAPQPPDVGSSDPLSLVCPSCQGRSPSYAS

SEQ ID NO: 16 - protein, 181 aa, synthetic construct
  REGION 1..181: note = FGF21 mutant protein
SHPIPDSSPLLQFGGQVRQRYLYTDDAQQTEAHLEIREDGTVGGAADQSPESLLQLKALKPGVIQILGVKTSRFLCQRPDGALYGSLHFDPEACSFRELLLEDGYNVYQSEAHGLPLHLPGQKSPHRDPAPRGPARFLPLPGLPPALPEPPGILAPQPPDVGSSDPLSLVGSQGRSPSYAS

SEQ ID NO: 17 - protein, 183 aa, synthetic construct
  REGION 1..183: note = FGF21 mutant protein
SHPIPDSSPLLQFGGQVRQRYLYTDDAQQTEAHLEIREDGTVGGAADQSPESLLQLKALKPGVIQILGVKTSRFLCQRPDGALYGSLHFDPEACSFRELLLEDGYNVYQSEAHGLPLHLPGQKSPHRDPAPRGPARFLPLPGLPPALPEPPGILAPQPPDVGSSDPLSLVCPGCQGRSPSYAS

SEQ ID NO: 18 - protein, 182 aa, synthetic construct
  REGION 1..182: note = FGF21 mutant protein
SHPIPDSSPLLQFGGQVRQRYLYTDDAQQTEAHLEIREDGTVGGAADQSPESLLQLKALKPGVIQILGVKTSRFLCQRPDGALYGSLHFDPEACSFRELLLEDGYNVYQSEAHGLPLHLPGQKSPHRDPAPRGPARFLPLPGLPPALPEPPGILAPQPPDVGSSDPLSLVCPCQGRSPSYAS

SEQ ID NO: 19 - protein, 182 aa, synthetic construct
  REGION 1..182: note = FGF21 mutant protein
SHPIPDSSPLLQFGGQVRQRYLYTDDAQQTEAHLEIREDGTVGGAADQSPESLLQLKALKPGVIQILGVKTSRFLCQRPDGALYGSLHFDPEACSFRELLLEDGYNVYQSEAHGLPLHLPGQKSPHRDPAPRGPARFLPLPGLPPALPEPPGILAPQPPDVGSSDPLSLVCPSCGRSPSYAS

SEQ ID NO: 20 - protein, 183 aa, synthetic construct
  REGION 1..183: note = FGF21 mutant protein
SHPIPDSSPLLQFGGQVRQRYLYTDDAQQTEAHLEIREDGTVGGAADQSPESLLQLKALKPGVIQILGVKTSRFLCQRPDGALYGSLHFDPEACSFRELLLEDGYNVYQSEAHGLPLHLPGQKSPHRDPAPRGPARFLPLPGLPPALPEPPGILAPQPPDVGSSDPLSLVCPACQGRSPSYAS

SEQ ID NO: 21 - protein, 183 aa, synthetic construct
  REGION 1..183: note = FGF21 mutant protein
SHPIPDSSPLLQFGGQVRQRYLYTDDAQQTEAHLEIREDGTVGGAADQSPESLLQLKALKPGVIQILGVKTSRFLCQRPDGALYGSLHFDPEACSFRELLLEDGYNVYQSEAHGLPLHLPGQKSPHRDPAPRGPARFLPLPGLPPALPEPPGILAPQPPDVGSSDPLSLVCPSCQGRSPSYAS

SEQ ID NO: 22 - protein, 181 aa, synthetic construct
  REGION 1..181: note = FGF21 mutant protein
GHPIPDSSPLLQFGGQVRQRYLYTDDAQQTEAHLEIREDGTVGGAADQSPESLLQLKALKPGVIQILGVKTSRFLCQRPDGALYGSLHFDPEACSFRELLLEDGYNVYQSEAHGLPLHLPGQKSPHRDPAPRGPARFLPLPGLPPALPEPPGILAPQPPDVGSSDPLSLVGSQGRSPSYAS

SEQ ID NO: 23 - protein, 183 aa, synthetic construct
  REGION 1..183: note = FGF21 mutant protein
GHPIPDSSPLLQFGGQVRQRYLYTDDAQQTEAHLEIREDGTVGGAADQSPESLLQLKALKPGVIQILGVKTSRFLCQRPDGALYGSLHFDPEACSFRELLLEDGYNVYQSEAHGLPLHLPGQKSPHRDPAPRGPARFLPLPGLPPALPEPPGILAPQPPDVGSSDPLSLVCPGCQGRSPSYAS

SEQ ID NO: 24 - protein, 182 aa, synthetic construct
  REGION 1..182: note = FGF21 mutant protein
GHPIPDSSPLLQFGGQVRQRYLYTDDAQQTEAHLEIREDGTVGGAADQSPESLLQLKALKPGVIQILGVKTSRFLCQRPDGALYGSLHFDPEACSFRELLLEDGYNVYQSEAHGLPLHLPGQKSPHRDPAPRGPARFLPLPGLPPALPEPPGILAPQPPDVGSSDPLSLVCPCQGRSPSYAS

SEQ ID NO: 25 - protein, 182 aa, synthetic construct
  REGION 1..182: note = FGF21 mutant protein
GHPIPDSSPLLQFGGQVRQRYLYTDDAQQTEAHLEIREDGTVGGAADQSPESLLQLKALKPGVIQILGVKTSRFLCQRPDGALYGSLHFDPEACSFRELLLEDGYNVYQSEAHGLPLHLPGQKSPHRDPAPRGPARFLPLPGLPPALPEPPGILAPQPPDVGSSDPLSLVCPSCGRSPSYAS

SEQ ID NO: 26 - protein, 183 aa, synthetic construct
  REGION 1..183: note = FGF21 mutant protein
GHPIPDSSPLLQFGGQVRQRYLYTDDAQQTEAHLEIREDGTVGGAADQSPESLLQLKALKPGVIQILGVKTSRFLCQRPDGALYGSLHFDPEACSFRELLLEDGYNVYQSEAHGLPLHLPGQKSPHRDPAPRGPARFLPLPGLPPALPEPPGILAPQPPDVGSSDPLSLVCPACQGRSPSYAS

SEQ ID NO: 27 - protein, 183 aa, synthetic construct
  REGION 1..183: note = FGF21 mutant protein
GHPIPDSSPLLQFGGQVRQRYLYTDDAQQTEAHLEIREDGTVGGAADQSPESLLQLKALKPGVIQILGVKTSRFLCQRPDGALYGSLHFDPEACSFRELLLEDGYNVYQSEAHGLPLHLPGQKSPHRDPAPRGPARFLPLPGLPPALPEPPGILAPQPPDVGSSDPLSLVCPSCQGRSPSYAS